European Patent Application EP 4 282 965 A1, published November 29, 2023. Title: ASPARTATE KINASE GENE EXPRESSION REGULATORY SEQUENCE AND USE THEREOF. Applicant: Tianjin Institute of Industrial Biotechnology, Chinese Academy of Sciences. The sequence listing filed with the application follows.

SEQUENCE LISTING (4 sequences)

SEQ ID NO: 1 - DNA, 373 bp, Artificial Sequence
gaaaacccaggattgctttgtgcactcctgggttttcactttgttaagcagttttggggaaaagtgcaaagtttgcaaagtttagaaatattttaagaggtaagatgtctgcaggtggaagcgtttaaatgcgttaaacttggccaaatgtggcaacctttgcaaggtgaaaaactggggcggggttagatcctggggggtttatttcattcactttggcttgaagtcgtgcaggtcaggggagtgttgcccgaaaacattgagaggaaaacaaaaaccgggccttgattgtaagataagacatttagtataattagacgcagtgactgctatcacccttggcggtctcttgttgaaaggaataattactcta

SEQ ID NO: 2 - DNA, 370 bp, Artificial Sequence
gaaaacccaggattgctttgtgcactcctgggttttcactttgttaagcagttttggggaaaagtgcaaagtttgcaaagtttagaaatattttaagaggtaagatgtctgcaggtggaagcgtttaaatgcgttaaacttggccaaatgtggcaacctttgcaaggtgaaaaactggggcggggttagatcctggggggtttatttcattcactttggcttgaagtcgtgcaggtcaggggagtgttgcccgaaaacattgagaggaaaacaaaaaccgggccttgattgtaagataagacatttagtataattagacgcagtgactgctatcacccttggcggtctcttgttgaaaggaataaaggtg

SEQ ID NO: 3 - DNA, 370 bp, Artificial Sequence
gaaaacccaggattgctttgtgcactcctgggttttcactttgttaagcagttttggggaaaagtgcaaagtttgcaaagtttagaaatattttaagaggtaagatgtctgcaggtggaagcgtttaaatgcgttaaacttggccaaatgtggcaacctttgcaaggtgaaaaactggggcggggttagatcctggggggtttatttcattcactttggcttgaagtcgtgcaggtcaggggagtgttgcccgaaaacattgagaggaaaacaaaaaccgggccttgattgtaagataagacatttagtataattagacgcagtgactgctatcacccttggcggtctcttgttgaaaggaataatcgtg

SEQ ID NO: 4 - DNA, 370 bp, Artificial Sequence
gaaaacccaggattgctttgtgcactcctgggttttcactttgttaagcagttttggggaaaagtgcaaagtttgcaaagtttagaaatattttaagaggtaagatgtctgcaggtggaagcgtttaaatgcgttaaacttggccaaatgtggcaacctttgcaaggtgaaaaactggggcggggttagatcctggggggtttatttcattcactttggcttgaagtcgtgcaggtcaggggagtgttgcccgaaaacattgagaggaaaacaaaaaccgggccttgattgtaagataagacatttagtataattagacgcagtgactgctatcacccttggcggtctcttgttgaaaggaataattttg